European Patent Application EP 4 574 840 A1, published June 25, 2025. Title: 糸状菌を用いた免疫グロブリンまたは多量体免疫グロブリンの製造方法. Applicant: 国立大学法人　東京大学. Application WO, filed August 14, 2023. The sequence listing filed with the application follows.

SEQUENCE LISTING (16 sequences)

SEQ ID NO: 1 - protein, 134 aa, Mus musculus
MKCSWIIFFLMAVVTGVNSEVQLQQSGSELVKSGASVKLSCTVSGFNFTDYYIHWVRQRTEQGLEWIGRIDPENDETTYAPKFQGKATMTADTSSNTAYLQLTSLTSEDTAVYYCARSTVLDYWGHGTTLTVSS

SEQ ID NO: 2 - protein, 131 aa, synthetic construct
MKLPVRLLVLMFWIPGFSSDVLMTQSPASLSVSLGDRATISCRASQSIVHTNGNTYLEWYLQKPGQSPKLLIYKVSNRFSGVPDRFSGSGSGTDFILKISRVEAEDLGVYYCFQGSHVPPTFGGGTKLEVK

SEQ ID NO: 3 - DNA, 1443 bp, synthetic construct
  source 1..1443: mol_type = other DNA
atgatggtcgcgtggtggtctctatttctgtacggccttcaggtcgcggcacctgctttggctgaggttcagctccagcagtctggttccgagcttgtcaagtctggtgcctccgtcaagctttcctgcaccgtttctggtttcaacttcactgactactacatccactgggtccgtcagcgtactgaacagggtctcgaatggattggtcgtattgaccctgagaacgacgaaactacctatgcccccaagttccagggtaaggccactatgaccgctgacacctcttccaacaccgcctacctccagctcacctccctcacctctgaggacactgccgtctactactgcgctcgttctactgtccttgactactggggtcacggcaccactctcaccgtctcctccgagtctgcccgtaaccccaccatctaccccctcactctcccccgtgctctctcctccgaccccgttatcatcggttgcctcattcacgattacttcccctccggcactatgaacgtcacctggggtaagtccggtaaggatatcaccaccgttaacttcccccctgccctcgcctctggtggtggttacaccatgtcctcccagcttaccctccccgctgtcgagtgccccgagggtgaatccgttaagtgctccgtccaacacgactctaacgccgttcaagaacttgatgtcaagtgctctggtcctccccctccctgtcctccctgtcctccctcctgccacccctccctctccctccagcgtcccgctcttgaggacctcctcctcggttccgatgcctccctcacttgtactctcaacggcctccgtaaccctgagggtgctgtcttcacctgggagccctccactggtaaggatgctgttcagaagaaggctgtccagaactcctgcggctgctactccgtctcctccgttctccctggttgtgctgagcgctggaactctggcgcttccttcaagtgcactgttacccaccctgagtctgacacccttactggtaccattgccaagatcaccgtcaacaccttccctccccaggtccacctccttcctcctccctccgaggagctcgccctcaacgagctcgtctccctcacctgcctcgtccgtgctttcaaccctaaggaggttctcgtccgttggctccacggtaacgaggagctctcccccgaatcctaccttgtcttcgagccccttaaggagcccggcgagggtgccaccacctacctcgttacttccgtccttcgtgtttccgctgaactctggaagcagggtgaccagtactcctgcatggttggtcacgaggcccttcccatgaacttcacccagaagaccatcgaccgtctctccggtaagcccaccaacgtctccgtctctgtcatcatgtccgagggtgatggcatctgctactga

SEQ ID NO: 4 - protein, 480 aa, synthetic construct
MMVAWWSLFLYGLQVAAPALAEVQLQQSGSELVKSGASVKLSCTVSGFNFTDYYIHWVRQRTEQGLEWIGRIDPENDETTYAPKFQGKATMTADTSSNTAYLQLTSLTSEDTAVYYCARSTVLDYWGHGTTLTVSSESARNPTIYPLTLPRALSSDPVIIGCLIHDYFPSGTMNVTWGKSGKDITTVNFPPALASGGGYTMSSQLTLPAVECPEGESVKCSVQHDSNAVQELDVKCSGPPPPCPPCPPSCHPSLSLQRPALEDLLLGSDASLTCTLNGLRNPEGAVFTWEPSTGKDAVQKKAVQNSCGCYSVSSVLPGCAERWNSGASFKCTVTHPESDTLTGTIAKITVNTFPPQVHLLPPPSEELALNELVSLTCLVRAFNPKEVLVRWLHGNEELSPESYLVFEPLKEPGEGATTYLVTSVLRVSAELWKQGDQYSCMVGHEALPMNFTQKTIDRLSGKPTNVSVSVIMSEGDGICY

SEQ ID NO: 5 - DNA, 723 bp, synthetic construct
  source 1..723: mol_type = other DNA
atgatggtcgcgtggtggtctctatttctgtacggccttcaggtcgcggcacctgctttggctgacgttctcatgacccagtctcccgcctccctctctgtctcccttggtgaccgtgccaccatctcttgccgtgcttcccagtccatcgtccacactaacggtaacacctacctcgagtggtacctccagaagcccggtcagtctcccaagctccttatctacaaggtttccaaccgtttctctggtgtccccgaccgtttctccggttccggttctggtaccgatttcatcctcaagatctcccgtgtcgaggctgaggaccttggtgtttactactgcttccagggttcccacgttcctcctactttcggtggtggtaccaagcttgaggtcaagcgtgctgacgctgcccccactgtctccatcttccccccctcctccgagcagctcacctctggtggtgcctccgtcgtctgcttcctcaacaacttctaccccaaggacatcaacgtcaagtggaagattgatggctccgaacgtcagaacggcgtccttaactcctggactgaccaggactccaaggactccacctactccatgtcctccaccctcactctcaccaaggacgagtacgaacgtcacaactcctacacctgcgaggccactcacaagacctccacttcccccattgtcaagtccttcaaccgtaacgagtgctga

SEQ ID NO: 6 - protein, 240 aa, synthetic construct
MMVAWWSLFLYGLQVAAPALADVLMTQSPASLSVSLGDRATISCRASQSIVHTNGNTYLEWYLQKPGQSPKLLIYKVSNRFSGVPDRFSGSGSGTDFILKISRVEAEDLGVYYCFQGSHVPPTFGGGTKLEVKRADAAPTVSIFPPSSEQLTSGGASVVCFLNNFYPKDINVKWKIDGSERQNGVLNSWTDQDSKDSTYSMSSTLTLTKDEYERHNSYTCEATHKTSTSPIVKSFNRNEC

SEQ ID NO: 7 - DNA, 480 bp, synthetic construct
  source 1..480: mol_type = other DNA
atgatggtcgcgtggtggtctctatttctgtacggccttcaggtcgcggcacctgctttggctggtgacgacgaagccaccatccttgctgacaacaagtgcatgtgtacccgtgttacctcccgtatcatcccctccaccgaggatcccaacgaggacatcgtcgagcgtaacatccgtatcgttgtccccctcaacaaccgtgagaacatctccgatcccacctcccccctccgtcgtaacttcgtctaccacctctccgacgtctgtaagaagtgcgatcccgtcgaagtcgagctcgaagatcaggttgttactgccacccagtccaacatctgcaacgaagacgatggtgttcctgagacctgctacatgtacgaccgtaacaagtgctacaccactatggtcccccttcgttaccacggtgagaccaagatggtccaggctgccctcacccccgattcctgctaccctgactag

SEQ ID NO: 8 - protein, 159 aa, synthetic construct
MMVAWWSLFLYGLQVAAPALAGDDEATILADNKCMCTRVTSRIIPSTEDPNEDIVERNIRIVVPLNNRENISDPTSPLRRNFVYHLSDVCKKCDPVEVELEDQVVTATQSNICNEDDGVPETCYMYDRNKCYTTMVPLRYHGETKMVQAALTPDSCYPD

SEQ ID NO: 9 - DNA, 1710 bp, synthetic construct
  source 1..1710: mol_type = other DNA
atgatggtcgcgtggtggtctctatttctgtacggccttcaggtcgcggcacctgctttggctgaggttcagctccagcagtctggttccgagcttgtcaagtctggtgcctccgtcaagctttcctgcaccgtttctggtttcaacttcactgactactacatccactgggtccgtcagcgtactgaacagggtctcgaatggattggtcgtattgaccctgagaacgacgaaactacctatgcccccaagttccagggtaaggccactatgaccgctgacacctcttccaacaccgcctacctccagctcacctccctcacctctgaggacactgccgtctactactgcgctcgttctactgtccttgactactggggtcacggcaccactctcaccgtctcctccgagtctgcccgtaaccccaccatctaccccctcactctcccccgtgctctctcctccgaccccgttatcatcggttgcctcattcacgattacttcccctccggcactatgaacgtcacctggggtaagtccggtaaggatatcaccaccgttaacttcccccctgccctcgcctctggtggtggttacaccatgtcctcccagcttaccctccccgctgtcgagtgccccgagggtgaatccgttaagtgctccgtccaacacgactctaacgccgttcaagaacttgatgtcaagtgctctggtcctccccctccctgtcctccctgtcctccctcctgccacccctccctctccctccagcgtcccgctcttgaggacctcctcctcggttccgatgcctccctcacttgtactctcaacggcctccgtaaccctgagggtgctgtcttcacctgggagccctccactggtaaggatgctgttcagaagaaggctgtccagaactcctgcggctgctactccgtctcctccgttctccctggttgtgctgagcgctggaactctggcgcttccttcaagtgcactgttacccaccctgagtctgacacccttactggtaccattgccaagatcaccgtcaacaccttccctccccaggtccacctccttcctcctccctccgaggagctcgccctcaacgagctcgtctccctcacctgcctcgtccgtgctttcaaccctaaggaggttctcgtccgttggctccacggtaacgaggagctctcccccgaatcctaccttgtcttcgagccccttaaggagcccggcgagggtgccaccacctacctcgttacttccgtccttcgtgtttccgctgaactctggaagcagggtgaccagtactcctgcatggttggtcacgaggcccttcccatgaacttcacccagaagaccatcgaccgtctctccggtaagcccaccaacgtctccgtctctgtcatcatgtccgagggtgatggcatctgctactcctccgctgacgatgccgctgctgatgctgccgccgccgatgatgctgctgctgacgacgccgctgctgacgcttccaactccgagggtcagatccccctcggtggtgacctcgccccccagatgctccgtgaacttcaggagactaacgccgccctccaagacgtccgtgagctccttcgtcagcaggtcaaggagatcaccttcctcaagaacactgtcatggaatgtgatgcttgcggtatgcagcccgctcgcactcccggctga

SEQ ID NO: 10 - protein, 569 aa, synthetic construct
MMVAWWSLFLYGLQVAAPALAEVQLQQSGSELVKSGASVKLSCTVSGFNFTDYYIHWVRQRTEQGLEWIGRIDPENDETTYAPKFQGKATMTADTSSNTAYLQLTSLTSEDTAVYYCARSTVLDYWGHGTTLTVSSESARNPTIYPLTLPRALSSDPVIIGCLIHDYFPSGTMNVTWGKSGKDITTVNFPPALASGGGYTMSSQLTLPAVECPEGESVKCSVQHDSNAVQELDVKCSGPPPPCPPCPPSCHPSLSLQRPALEDLLLGSDASLTCTLNGLRNPEGAVFTWEPSTGKDAVQKKAVQNSCGCYSVSSVLPGCAERWNSGASFKCTVTHPESDTLTGTIAKITVNTFPPQVHLLPPPSEELALNELVSLTCLVRAFNPKEVLVRWLHGNEELSPESYLVFEPLKEPGEGATTYLVTSVLRVSAELWKQGDQYSCMVGHEALPMNFTQKTIDRLSGKPTNVSVSVIMSEGDGICYSSADDAAADAAAADDAAADDAAADASNSEGQIPLGGDLAPQMLRELQETNAALQDVRELLRQQVKEITFLKNTVMECDACGMQPARTPG

SEQ ID NO: 11 - DNA, 723 bp, synthetic construct; identical to SEQ ID NO: 5
  source 1..723: mol_type = other DNA

SEQ ID NO: 12 - protein, 240 aa, synthetic construct; identical to SEQ ID NO: 6

SEQ ID NO: 13 - protein, 548 aa, synthetic construct
EVQLQQSGSELVKSGASVKLSCTVSGFNFTDYYIHWVRQRTEQGLEWIGRIDPENDETTYAPKFQGKATMTADTSSNTAYLQLTSLTSEDTAVYYCARSTVLDYWGHGTTLTVSSESARNPTIYPLTLPRALSSDPVIIGCLIHDYFPSGTMNVTWGKSGKDITTVNFPPALASGGGYTMSSQLTLPAVECPEGESVKCSVQHDSNAVQELDVKCSGPPPPCPPCPPSCHPSLSLQRPALEDLLLGSDASLTCTLNGLRNPEGAVFTWEPSTGKDAVQKKAVQNSCGCYSVSSVLPGCAERWNSGASFKCTVTHPESDTLTGTIAKITVNTFPPQVHLLPPPSEELALNELVSLTCLVRAFNPKEVLVRWLHGNEELSPESYLVFEPLKEPGEGATTYLVTSVLRVSAELWKQGDQYSCMVGHEALPMNFTQKTIDRLSGKPTNVSVSVIMSEGDGICYSSADDAAADAAAADDAAADDAAADASNSEGQIPLGGDLAPQMLRELQETNAALQDVRELLRQQVKEITFLKNTVMECDACGMQPARTPG

SEQ ID NO: 14 - protein, 548 aa, synthetic construct
EVQLQQSGSELVKSGASVKLSCTVSGFNFTDYYIHWVRQRTEQGLEWIGRIDPENDETTYAPKFQGKATMTADTSSNTAYLQLTSLTSEDTAVYYCARSTVLDYWGHGTTLTVSSESARNPTIYPLTLPRALSSDPVIIGCLIHDYFPSGTMNVTWGKSGKDITTVNFPPALASGGGYTMSSQLTLPAVECPEGESVKCSVQHDSNAVQELDVKCSGPPPPCPPCPPSCHPSLSLQRPALEDLLLGSDASLTCTLNGLRNPEGAVFTWEPSTGKDAVQKKAVQNSCGCYSVSSVLPGCAERWNSGASFKCTVTHPESDTLTGTIAKITVNTFPPQVHLLPPPSEELALNELVSLTCLVRAFNPKEVLVRWLHGNEELSPESYLVFEPLKEPGEGATTYLVTSVLRVSAELWKQGDQYSCMVGHEALPMNFTQKTIDRLSGKPTNVSVSVIMSEGDGICYSSADDAKKDAAAADDKKADDAKKDASNSEGQIPLGGDLAPQMLRELQETNAALQDVRELLRQQVKEITFLKNTVMECDACGMQPARTPG

SEQ ID NO: 15 - protein, 522 aa, synthetic construct
EVQLQQSGSELVKSGASVKLSCTVSGFNFTDYYIHWVRQRTEQGLEWIGRIDPENDETTYAPKFQGKATMTADTSSNTAYLQLTSLTSEDTAVYYCARSTVLDYWGHGTTLTVSSESARNPTIYPLTLPRALSSDPVIIGCLIHDYFPSGTMNVTWGKSGKDITTVNFPPALASGGGYTMSSQLTLPAVECPEGESVKCSVQHDSNAVQELDVKCSGPPPPCPPCPPSCHPSLSLQRPALEDLLLGSDASLTCTLNGLRNPEGAVFTWEPSTGKDAVQKKAVQNSCGCYSVSSVLPGCAERWNSGASFKCTVTHPESDTLTGTIAKITVNTFPPQVHLLPPPSEELALNELVSLTCLVRAFNPKEVLVRWLHGNEELSPESYLVFEPLKEPGEGATTYLVTSVLRVSAELWKQGDQYSCMVGHEALPMNFTQKTIDRLSGKPTNVSVSVIMSEGDGICYNSEGQIPLGGDLAPQMLRELQETNAALQDVRELLRQQVKEITFLKNTVMECDACGMQPARTPG

SEQ ID NO: 16 - protein, 504 aa, synthetic construct
EVQLQQSGSELVKSGASVKLSCTVSGFNFTDYYIHWVRQRTEQGLEWIGRIDPENDETTYAPKFQGKATMTADTSSNTAYLQLTSLTSEDTAVYYCARSTVLDYWGHGTTLTVSSESARNPTIYPLTLPRALSSDPVIIGCLIHDYFPSGTMNVTWGKSGKDITTVNFPPALASGGGYTMSSQLTLPAVECPEGESVKCSVQHDSNAVQELDVKCSGPPPPCPPCPPSCHPSLSLQRPALEDLLLGSDASLTCTLNGLRNPEGAVFTWEPSTGKDAVQKKAVQNSCGCYSVSSVLPGCAERWNSGASFKCTVTHPESDTLTGTIAKITVNTFPPQVHLLPPPSEELALNELVSLTCLVRAFNPKEVLVRWLHGNEELSPESYLVFEPLKEPGEGATTYLVTSVLRVSAELWKQGDQYSCMVGHEALPMNFTQKTIDRLSGKNSEGQIPLGGDLAPQMLRELQETNAALQDVRELLRQQVKEITFLKNTVMECDACGMQPARTPG